European Patent Specification EP 4 015 646 B1, published December 27, 2023. Title: NUCLEIC ACID SAMPLE PROCESSING METHOD, SEQUENCING METHOD AND KIT. Applicant: GeneMind Biosciences Company Limited. Application PCT/CN2020/108420. The sequence listing filed with the application follows.

SEQUENCE LISTING (8 sequences)

SEQ ID NO: 1 - DNA, 20 bp, Artificial Sequence
  artificial sequence
  misc_feature (1)..(20): adapter
agatgtgtataagagacagt

SEQ ID NO: 2 - DNA, 54 bp, Artificial Sequence
  artificial sequence
  misc_feature (1)..(54): adapter
actgtctcttatacacatctgagtggaactggatggtcgcaggtatcaaggatt

SEQ ID NO: 3 - DNA, 51 bp, Artificial Sequence
  artificial sequence
  misc_feature (1)..(51): adapter
ctgtctcttatacacatctgagtggaactggatggtcgcaggtatcaagga

SEQ ID NO: 4 - DNA, 33 bp, Artificial Sequence
  artificial sequence
  misc_feature (1)..(33): adapter
acactctttccctacacgacgctcttccgatct

SEQ ID NO: 5 - DNA, 31 bp, Artificial Sequence
  artificial sequence
  misc_feature (1)..(31): adapter
gatcggaagagcacacgtctgaactccagtc

SEQ ID NO: 6 - DNA, 58 bp, Artificial Sequence
  artificial sequence
  misc_feature (1)..(58): primer
aatgatacggcgaccaccgagatctacactctttccctacacgacgctcttccgatct

SEQ ID NO: 7 - DNA, 34 bp, Artificial Sequence
  artificial sequence
  misc_feature (1)..(34): primer
gtgactggagttcagacgtgtgctcttccgatct

SEQ ID NO: 8 - DNA, 60 bp, Artificial Sequence
  artificial sequence
  misc_feature (1)..(60): probe
tttttttttttccttgatacctgcgaccatccagttccactcagatgtgtataagagaca